European Patent Application EP 4 800 029 A1, published September 2, 2026. Title: NOVEL CHEMOKINE-LIKE PROTEIN FRAGMENTS. Applicant: NEURACLE GENETICS INC. The sequence listing filed with the application follows.

SEQUENCE LISTING (184 sequences)

SEQ ID NO: 1 - protein, 8 aa, synthetic construct
  REGION 1..8: note = Human TAFA4 fragment 3.7
EGEDCKVL

SEQ ID NO: 2 - protein, 8 aa, synthetic construct
  REGION 1..8: note = Chicken TAFA4 fragment 3.7
DGEDCKVL

SEQ ID NO: 3 - protein, 8 aa, synthetic construct
  REGION 1..8: note = Komodo dragon TAFA4 fragment 3.7
EGEECKVL

SEQ ID NO: 4 - protein, 8 aa, synthetic construct
  REGION 1..8: note = Fish TAFA4 fragment 3.7
DGEECKAL

SEQ ID NO: 5 - protein, 8 aa, synthetic construct
  REGION 1..8: note = Human TAFA1 fragment 3.7
EGEECKTL

SEQ ID NO: 6 - protein, 8 aa, synthetic construct
  REGION 1..8: note = Human TAFA2 fragment 3.7
EGEECKVL

SEQ ID NO: 7 - protein, 8 aa, synthetic construct
  REGION 1..8: note = Frog TAFA2 fragment 3.7
EGEECKIL

SEQ ID NO: 8 - protein, 8 aa, synthetic construct
  REGION 1..8: note = Fish TAFA2 fragment 3.7
DGEECKVL

SEQ ID NO: 9 - protein, 8 aa, synthetic construct
  REGION 1..8: note = Human TAFA3 fragment 3.7
PGEECKVL

SEQ ID NO: 10 - protein, 8 aa, synthetic construct
  REGION 1..8: note = Rat TAFA3 fragment 3.7
LGEECKVL

SEQ ID NO: 11 - protein, 8 aa, synthetic construct
  REGION 1..8: note = Chicken TAFA3 fragment 3.7
AGEECKVL

SEQ ID NO: 12 - protein, 8 aa, synthetic construct
  REGION 1..8: note = Komodo dragon TAFA3 fragment 3.7
EGEECKVL

SEQ ID NO: 13 - protein, 8 aa, synthetic construct
  REGION 1..8: note = Frog TAFA3 fragment 3.7
EGEDCKVL

SEQ ID NO: 14 - protein, 8 aa, synthetic construct
  REGION 1..8: note = Fish TAFA3 fragment 3.7
DGEECKVL

SEQ ID NO: 15 - protein, 17 aa, synthetic construct
  REGION 1..17: note = Human TAFA4 fragment 2.5
GQVAGTTRAQPSCVEAS

SEQ ID NO: 16 - protein, 17 aa, synthetic construct
  REGION 1..17: note = Rabbit TAFA4 fragment 2.5
GQVAGTTQAQPSCVEAS

SEQ ID NO: 17 - protein, 17 aa, synthetic construct
  REGION 1..17: note = Mouse TAFA4 fragment 2.5
GQVAGTTRAQPSCVEAA

SEQ ID NO: 18 - protein, 17 aa, synthetic construct
  REGION 1..17: note = Fence lizard TAFA4 fragment 2.5
GQVAGTTRSQPSCVEAA

SEQ ID NO: 19 - protein, 17 aa, synthetic construct
  REGION 1..17: note = Gecko TAFA4 fragment 2.5
GQVAGTTRTQPSCVEAA

SEQ ID NO: 20 - protein, 17 aa, synthetic construct
  REGION 1..17: note = Human TAFA1 fragment 2.5
GKVAGTTRNRPSCVDAS

SEQ ID NO: 21 - protein, 17 aa, synthetic construct
  REGION 1..17: note = Fish TAFA1 fragment 2.5
GKVAGTTRNKPSCVDAS

SEQ ID NO: 22 - protein, 15 aa, synthetic construct
  REGION 1..15: note = Gecko TAFA1 fragment 2.5
GKVAGTTRNRPSCVD

SEQ ID NO: 23 - protein, 17 aa, synthetic construct
  REGION 1..17: note = Human TAFA2 fragment 2.5
GQVAGTTRAAPSCVDAS

SEQ ID NO: 24 - protein, 17 aa, synthetic construct
  REGION 1..17: note = Frog TAFA2 fragment 2.5
GQVAGTTRATPSCVDAS

SEQ ID NO: 25 - protein, 17 aa, synthetic construct
  REGION 1..17: note = Human TAFA3 fragment 2.5
GQVAGTTRAKPSCVDAS

SEQ ID NO: 26 - protein, 17 aa, synthetic construct
  REGION 1..17: note = Chicken TAFA3 fragment 2.5
GQVAGTTRAAPSCVDAS

SEQ ID NO: 27 - protein, 17 aa, synthetic construct
  REGION 1..17: note = Wall lizard TAFA3 fragment 2.5
GQVAGTTHAAPSCVDAS

SEQ ID NO: 28 - protein, 22 aa, synthetic construct
  REGION 1..22: note = Human TAFA4 fragment 7
IVIQKWWCHMNPCLEGEDCKVL

SEQ ID NO: 29 - protein, 22 aa, synthetic construct
  REGION 1..22: note = Rabbit TAFA4 fragment 7
IVAQKWWCHMNPCLEGEDCKVL

SEQ ID NO: 30 - protein, 22 aa, synthetic construct
  REGION 1..22: note = Rat TAFA4 fragment 7
IVIEKWWCHMDPCLEGEDCKVL

SEQ ID NO: 31 - protein, 22 aa, synthetic construct
  REGION 1..22: note = Mouse TAFA4 fragment 7
IVIEKWWCHMNPCLEGEDCKVL

SEQ ID NO: 32 - protein, 22 aa, synthetic construct
  REGION 1..22: note = Chicken TAFA4 fragment 7
IVLQKWWCHMNPCLDGEDCKVL

SEQ ID NO: 33 - protein, 22 aa, synthetic construct
  REGION 1..22: note = Komodo dragon TAFA4 fragment 7
IVVQKWWCHMNPCLEGEECKVL

SEQ ID NO: 34 - protein, 22 aa, synthetic construct
  REGION 1..22: note = Wall lizard TAFA4 fragment 7
IVIQKWWCHMNPCLDGEDCKVL

SEQ ID NO: 35 - protein, 22 aa, synthetic construct
  REGION 1..22: note = Fence lizard TAFA4 fragment 7
IVIQKWWCHMNPCLEGEECKVL

SEQ ID NO: 36 - protein, 22 aa, synthetic construct
  REGION 1..22: note = Gecko TAFA4 fragment 7
IVIQKWWCQMSPCLEGEECKVL

SEQ ID NO: 37 - protein, 22 aa, synthetic construct
  REGION 1..22: note = Frog TAFA4 fragment 7
IVIQKWWCHMNPCMEGEECKVL

SEQ ID NO: 38 - protein, 22 aa, synthetic construct
  REGION 1..22: note = Fish TAFA4 fragment 7
IVLQKWWCQMHPCLDGEECKAL

SEQ ID NO: 39 - protein, 22 aa, synthetic construct
  REGION 1..22: note = Human TAFA1 fragment 7
IVIGKWWCEMEPCLEGEECKTL

SEQ ID NO: 40 - protein, 22 aa, synthetic construct
  REGION 1..22: note = Human TAFA2 fragment 7
IVEQKWWCHMQPCLEGEECKVL

SEQ ID NO: 41 - protein, 22 aa, synthetic construct
  REGION 1..22: note = Gecko TAFA2 fragment 7
IVEQKWWCQMQPCLEGEECKVL

SEQ ID NO: 42 - protein, 22 aa, synthetic construct
  REGION 1..22: note = Frog TAFA2 fragment 7
IVEQKWWCHMQPCLEGEECKIL

SEQ ID NO: 43 - protein, 22 aa, synthetic construct
  REGION 1..22: note = Fish TAFA2 fragment 7
IVAQKWWCQMQPCMDGEECKVL

SEQ ID NO: 44 - protein, 22 aa, synthetic construct
  REGION 1..22: note = Human TAFA3 fragment 7
IVLQRWWCQMEPCLPGEECKVL

SEQ ID NO: 45 - protein, 22 aa, synthetic construct
  REGION 1..22: note = Pig TAFA3 fragment 7
IVLQKWWCQMEPCLPGEECKVL

SEQ ID NO: 46 - protein, 22 aa, synthetic construct
  REGION 1..22: note = Rat TAFA3 fragment 7
IVLQKWWCQMEPCLLGEECKVL

SEQ ID NO: 47 - protein, 22 aa, synthetic construct
  REGION 1..22: note = Chicken TAFA3 fragment 7
IVLQKWWCQMEPCLAGEECKVL

SEQ ID NO: 48 - protein, 22 aa, synthetic construct
  REGION 1..22: note = Komodo dragon TAFA3 fragment 7
IVLQKWWCQMQPCLEGEECKVL

SEQ ID NO: 49 - protein, 22 aa, synthetic construct
  REGION 1..22: note = Wall lizard TAFA3 fragment 7
IVLQKWWCQMQPCVEGEECKVL

SEQ ID NO: 50 - protein, 22 aa, synthetic construct
  REGION 1..22: note = Frog TAFA3 fragment 7
IVIQKWWCQMEPCLEGEDCKVL

SEQ ID NO: 51 - protein, 22 aa, synthetic construct
  REGION 1..22: note = Fish TAFA3 fragment 7
IVAQKWWCQMQPCVDGEECKVL

SEQ ID NO: 52 - protein, 29 aa, synthetic construct
  REGION 1..29: note = Human TAFA4 fragment 3
EGEDCKVLPDYSGWSCSSGNKVKTTKVTR

SEQ ID NO: 53 - protein, 29 aa, synthetic construct
  REGION 1..29: note = Rat TAFA4 fragment 3
EGEDCKVLPDSSGWSCSSGNKVKTTKVTR

SEQ ID NO: 54 - protein, 29 aa, synthetic construct
  REGION 1..29: note = Chicken TAFA4 fragment 3
DGEDCKVLPDYSGWSCSSGNKVKTTKVTR

SEQ ID NO: 55 - protein, 29 aa, synthetic construct
  REGION 1..29: note = Komodo dragon TAFA4 fragment 3
EGEECKVLPDYSGWSCSSGNKVKTTKVTR

SEQ ID NO: 56 - protein, 29 aa, synthetic construct
  REGION 1..29: note = Gecko TAFA4 fragment 3
EGEECKVLPDSSGWSCSSGNKVKTTKVTR

SEQ ID NO: 57 - protein, 29 aa, synthetic construct
  REGION 1..29: note = Frog TAFA4 fragment 3
EGEECKVLPDLTGWSCSSGNKIKTTKVTR

SEQ ID NO: 58 - protein, 29 aa, synthetic construct
  REGION 1..29: note = Fish TAFA4 fragment 3
DGEECKALPDLTGWSCSTGNKVKTTKVTR

SEQ ID NO: 59 - protein, 32 aa, synthetic construct
  REGION 1..32: note = Human TAFA4 fragment 5
RIEERSQTVKCSCFPGQVAGTTRAQPSCVEAS

SEQ ID NO: 60 - protein, 32 aa, synthetic construct
  REGION 1..32: note = Rabbit TAFA4 fragment 5
RIEERSQTVKCSCFPGQVAGTTQAQPSCVEAS

SEQ ID NO: 61 - protein, 32 aa, synthetic construct
  REGION 1..32: note = Mouse TAFA4 fragment 5
RIEERSQTVKCSCFPGQVAGTTRAQPSCVEAA

SEQ ID NO: 62 - protein, 32 aa, synthetic construct
  REGION 1..32: note = Komodo dragon TAFA4 fragment 5
RIEERSQTVKCSCLPGQVAGTTRAQPSCVEAA

SEQ ID NO: 63 - protein, 32 aa, synthetic construct
  REGION 1..32: note = Fence lizard TAFA4 fragment 5
RIEERSQTVKCSCFPGQVAGTTRSQPSCVEAA

SEQ ID NO: 64 - protein, 32 aa, synthetic construct
  REGION 1..32: note = Gecko TAFA4 fragment 5
RIEELSQTGNCSCLPGQVAGTTRTQPSCVEAA

SEQ ID NO: 65 - protein, 32 aa, synthetic construct
  REGION 1..32: note = Fish TAFA4 fragment 5
KIEERSQTVKCSCFPGQVAGTTRAQPSCVEAS

SEQ ID NO: 66 - protein, 32 aa, synthetic construct
  REGION 1..32: note = Human TAFA1 fragment 5
RIEERSQTVKCSCLPGKVAGTTRNRPSCVDAS

SEQ ID NO: 67 - protein, 30 aa, synthetic construct
  REGION 1..30: note = Gecko TAFA1 fragment 5
RIEERSQTVKCSCLPGKVAGTTRNRPSCVD

SEQ ID NO: 68 - protein, 32 aa, synthetic construct
  REGION 1..32: note = Fish TAFA1 fragment 5
KIEERSQTVKCSCLPGKVAGTTRNKPSCVDAS

SEQ ID NO: 69 - protein, 32 aa, synthetic construct
  REGION 1..32: note = Human TAFA2 fragment 5
KIEERSQTVKCSCFPGQVAGTTRAAPSCVDAS

SEQ ID NO: 70 - protein, 32 aa, synthetic construct
  REGION 1..32: note = Frog TAFA2 fragment 5
KIEERSQTVKCSCFPGQVAGTTRATPSCVDAS

SEQ ID NO: 71 - protein, 32 aa, synthetic construct
  REGION 1..32: note = Human TAFA3 fragment 5
RIEERSQTVKCSCFSGQVAGTTRAKPSCVDAS

SEQ ID NO: 72 - protein, 32 aa, synthetic construct
  REGION 1..32: note = Rabbit TAFA3 fragment 5
RIEERSQTVKCSCLSGQVAGTTRAKPSCVDAS

SEQ ID NO: 73 - protein, 32 aa, synthetic construct; identical to SEQ ID NO: 69
  REGION 1..32: note = Chicken TAFA3 fragment 5

SEQ ID NO: 74 - protein, 32 aa, synthetic construct
  REGION 1..32: note = Wall lizard TAFA3 fragment 5
KIEERSQTVKCSCFPGQVAGTTHAAPSCVDAS

SEQ ID NO: 75 - protein, 31 aa, synthetic construct
  REGION 1..31: note = Human TAFA4 fragment 2
GQVAGTTRAQPSCVEASIVIQKWWCHMNPCL

SEQ ID NO: 76 - protein, 31 aa, synthetic construct
  REGION 1..31: note = Rabbit TAFA4 fragment 2
GQVAGTTQAQPSCVEASIVAQKWWCHMNPCL

SEQ ID NO: 77 - protein, 31 aa, synthetic construct
  REGION 1..31: note = Rat TAFA4 fragment 2
GQVAGTTRAQPSCVEASIVIEKWWCHMDPCL

SEQ ID NO: 78 - protein, 31 aa, synthetic construct
  REGION 1..31: note = Mouse TAFA4 fragment 2
GQVAGTTRAQPSCVEAAIVIEKWWCHMNPCL

SEQ ID NO: 79 - protein, 31 aa, synthetic construct
  REGION 1..31: note = Chicken TAFA4 fragment 2
GQVAGTTRAQPSCVEASIVLQKWWCHMNPCL

SEQ ID NO: 80 - protein, 31 aa, synthetic construct
  REGION 1..31: note = Komodo dragon TAFA4 fragment 2
GQVAGTTRAQPSCVEAAIVVQKWWCHMNPCL

SEQ ID NO: 81 - protein, 31 aa, synthetic construct
  REGION 1..31: note = Wall lizard TAFA4 fragment 2
GQVAGTTRAQPSCVEAAIVIQKWWCHMNPCL

SEQ ID NO: 82 - protein, 31 aa, synthetic construct
  REGION 1..31: note = Fence lizard TAFA4 fragment 2
GQVAGTTRSQPSCVEAAIVIQKWWCHMNPCL

SEQ ID NO: 83 - protein, 31 aa, synthetic construct
  REGION 1..31: note = Gecko TAFA4 fragment 2
GQVAGTTRTQPSCVEAAIVIQKWWCQMSPCL

SEQ ID NO: 84 - protein, 31 aa, synthetic construct
  REGION 1..31: note = Frog TAFA4 fragment 2
GQVAGTTRAQPSCVEASIVIQKWWCHMNPCM

SEQ ID NO: 85 - protein, 31 aa, synthetic construct
  REGION 1..31: note = Fish TAFA4 fragment 2
GQVAGTTRAQPSCVEASIVLQKWWCQMHPCL

SEQ ID NO: 86 - protein, 105 aa, synthetic construct
  REGION 1..105: note = Recombinant human TAFA4
SQHLRGHAGHHQIKQGTCEVVAVHRCCNKNRIEERSQTVKCSCFPGQVAGTTRAQPSCVEASIVIQKWWCHMNPCLEGEDCKVLPDYSGWSCSSGNKVKTTKVTR

SEQ ID NO: 87 - protein, 93 aa, synthetic construct
  REGION 1..93: note = TAFA4_Homo sapiens
IKQGTCEVVAVHRCCNKNRIEERSQTVKCSCFPGQVAGTTRAQPSCVEASIVIQKWWCHMNPCLEGEDCKVLPDYSGWSCSSGNKVKTTKVTR

SEQ ID NO: 88 - protein, 91 aa, synthetic construct
  REGION 1..91: note = TAFA1_Homo sapiens
EGGTCEVIAAHRCCNKNRIEERSQTVKCSCLPGKVAGTTRNRPSCVDASIVIGKWWCEMEPCLEGEECKTLPDNSGWMCATGNKIKTTRIH

SEQ ID NO: 89 - protein, 91 aa, synthetic construct; identical to SEQ ID NO: 88
  REGION 1..91: note = TAFA1_Macaca fascicularis_isoform1

SEQ ID NO: 90 - protein, 91 aa, synthetic construct; identical to SEQ ID NO: 88
  REGION 1..91: note = TAFA1_Sus scrofa_isoform2

SEQ ID NO: 91 - protein, 91 aa, synthetic construct; identical to SEQ ID NO: 88
  REGION 1..91: note = TAFA1_Oryctolagus cuniculus_isoform1

SEQ ID NO: 92 - protein, 91 aa, synthetic construct; identical to SEQ ID NO: 88
  REGION 1..91: note = TAFA1_Rattus norvegicus_isoform1

SEQ ID NO: 93 - protein, 91 aa, synthetic construct; identical to SEQ ID NO: 88
  REGION 1..91: note = TAFA1_Mus musculus

SEQ ID NO: 94 - protein, 91 aa, synthetic construct; identical to SEQ ID NO: 88
  REGION 1..91: note = TAFA1_Gallus gallus_isoform2

SEQ ID NO: 95 - protein, 91 aa, synthetic construct
  REGION 1..91: note = TAFA1_Varanus komodoensis
EGGTCEVIAAHRCCNKNRIEERSQTVKCSCLPGKVAGTTRNRPSCVDASIVIGKWWCEMEPCLEGEECKTLPDNSGWMCATGNKVKTTRIH

SEQ ID NO: 96 - protein, 91 aa, synthetic construct; identical to SEQ ID NO: 95
  REGION 1..91: note = TAFA1_Podarcis muralis_isoform1

SEQ ID NO: 97 - protein, 91 aa, synthetic construct; identical to SEQ ID NO: 95
  REGION 1..91: note = TAFA1_Sceloporus undulatus_isoform1

SEQ ID NO: 98 - protein, 92 aa, synthetic construct
  REGION 1..92: note = TAFA1_Xenopus tropicalis_isoform1
IEGGTCEVIAAHRCCNKNRIEERSQTVKCSCLPGKVAGTTRNRPSCVDASIVIGKWWCEMEPCLEGEECKTLPDNSGWMCATGNKIKTTRFQ

SEQ ID NO: 99 - protein, 92 aa, synthetic construct
  REGION 1..92: note = TAFA1_Xenopus tropicalis_isoform2
IEGGTCEVIAAHRCCNKNRIEERSQTVKCSCLPGKVAGTTRNRPSCVDASIVIGKWWCEMEPCLEGEECKTLPDNSGWMCATGNKIKTTRIH

SEQ ID NO: 100 - protein, 93 aa, synthetic construct
  REGION 1..93: note = TAFA1_Danio rerio_isoform1
LEGGTCEVIAAHRCCNKNKIEERSQTVKCSCLPGKVAGTTRNKPSCVDASIVIGKWWCEMEPCLEGEECKTLPDNSGWMCYSGNKIKTTRGNI

SEQ ID NO: 101 - protein, 93 aa, synthetic construct
  REGION 1..93: note = TAFA1_Danio rerio_isoform2
LEGGTCEVIAAHRCCNKNKIEERSQTVKCSCLPGKVAGTTRNKPSCVDASIVIGKWWCEMEPCLEGEECKTLPDNSGWMCYSGNKIKTTRNTH

SEQ ID NO: 102 - protein, 93 aa, synthetic construct
  REGION 1..93: note = TAFA2_Homo sapiens
VKTGTCEVVALHRCCNKNKIEERSQTVKCSCFPGQVAGTTRAAPSCVDASIVEQKWWCHMQPCLEGEECKVLPDRKGWSCSSGNKVKTTRVTH

SEQ ID NO: 103 - protein, 93 aa, synthetic construct; identical to SEQ ID NO: 102
  REGION 1..93: note = TAFA2_Macaca fascicularis

SEQ ID NO: 104 - protein, 93 aa, synthetic construct; identical to SEQ ID NO: 102
  REGION 1..93: note = TAFA2_Sus scrofa

SEQ ID NO: 105 - protein, 93 aa, synthetic construct; identical to SEQ ID NO: 102
  REGION 1..93: note = TAFA2_Oryctolagus cuniculus

SEQ ID NO: 106 - protein, 93 aa, synthetic construct
  REGION 1..93: note = TAFA2_Rattus norvegicus_isoform1
VRTGTCEVVALHRCCNKNKIEERSQTVKCSCFPGQVAGTTRAAPSCVDASIVEQKWWCHMQPCLEGEECKVLPDRKGWSCSSGNKVKTTRANV

SEQ ID NO: 107 - protein, 93 aa, synthetic construct
  REGION 1..93: note = TAFA2_Rattus norvegicus_isoform2
VRTGTCEVVALHRCCNKNKIEERSQTVKCSCFPGQVAGTTRAAPSCVDASIVEQKWWCHMQPCLEGEECKVLPDRKGWSCSSGNKVKTTRVTH

SEQ ID NO: 108 - protein, 93 aa, synthetic construct; identical to SEQ ID NO: 107
  REGION 1..93: note = TAFA2_Mus musculus_isoform1

SEQ ID NO: 109 - protein, 93 aa, synthetic construct
  REGION 1..93: note = TAFA2_Gallus gallus_isoform1
VKTGTCEVVALHRCCNKNKIEERSQTVKCSCFPGQVAGTTRAAPSCVDASIVEQKWWCHMQPCLEGEECKVLPDRKGWSCSSGNKVKTTRANV

SEQ ID NO: 110 - protein, 93 aa, synthetic construct
  REGION 1..93: note = TAFA2_Gallus gallus_isoform2
VKTGTCEVVALHRCCNKNKIEERSQTVKCSCFPGQVAGTTRAAPSCVDASIVEQKWWCHMQPCLEGEECKVLPDRKGWSCSSGNKVKTTRVTR

SEQ ID NO: 111 - protein, 93 aa, synthetic construct
  REGION 1..93: note = TAFA2_Varanus komodoensis
VKTGTCEVVALHRCCNKNKIEERSQTVKCSCFPGQVAGTTRAAPSCVDASIVEQKWWCHMQPCLEGEECKVLPDRKGWSCSSGNKVKTTRVSK

SEQ ID NO: 112 - protein, 91 aa, synthetic construct
  REGION 1..91: note = TAFA2_Podarcis muralis
VKTGTCEVVALHRCCNKNKIEERSQTVKCSCFPGQVAGTTRAAPSCVDASIVEQKWWCHMQPCLEGEECKVLPDRKGWSCSSGNKVKTTRM

SEQ ID NO: 113 - protein, 93 aa, synthetic construct; identical to SEQ ID NO: 110
  REGION 1..93: note = TAFA2_Podarcis muralis

SEQ ID NO: 114 - protein, 93 aa, synthetic construct; identical to SEQ ID NO: 110
  REGION 1..93: note = TAFA2_Sceloporus undulatus

SEQ ID NO: 115 - protein, 92 aa, synthetic construct
  REGION 1..92: note = TAFA2_Gekko japonicus
VKTGTCEVVALHRCCNKNKIEERSQTVKCSCFPGQVAGTTRAAPSCVDASIVEQKWWCQMQPCLEGEECKVLPDRKGWSCSSGNKVKTTRAN

SEQ ID NO: 116 - protein, 93 aa, synthetic construct
  REGION 1..93: note = TAFA2_Xenopus tropicalis
VRTGTCEVVALHRCCNKNKIEERSQTVKCSCFPGQVAGTTRATPSCVDASIVEQKWWCHMQPCLEGEECKILPDQKGWSCASGNKVKTTKVTR

SEQ ID NO: 117 - protein, 93 aa, synthetic construct
  REGION 1..93: note = TAFA2_Danio rerio
VKAGTCEVIAAHRCCNKNKIEERSQTVKCSCFPGQVAGTTRAAPSCVDASIVAQKWWCQMQPCMDGEECKVLPDLKGWSCSTGNKVKTTKVTR

SEQ ID NO: 118 - protein, 93 aa, synthetic construct
  REGION 1..93: note = TAFA3_Homo sapiens_isoform1
VQQGTCEVIAAHRCCNRNRIEERSQTVKCSCFSGQVAGTTRAKPSCVDASIVLQRWWCQMEPCLPGEECKVLPDLSGWSCSSGHKVKTTKVTR

SEQ ID NO: 119 - protein, 93 aa, synthetic construct; identical to SEQ ID NO: 118
  REGION 1..93: note = TAFA3_Macaca fascicularis_isoform3

SEQ ID NO: 120 - protein, 93 aa, synthetic construct
  REGION 1..93: note = TAFA3_Sus scrofa_isoform2
VKQGTCEVIAAHRCCNRNRIEERSQTVKCSCFSGQVAGTTRAKPSCVDASIVLQKWWCQMEPCLPGEECKVLPDLSGWSCSSGHKVKTTKVTR

SEQ ID NO: 121 - protein, 93 aa, synthetic construct
  REGION 1..93: note = TAFA3_Oryctolagus cuniculus_isoform2
VKQGTCEVIAAHRCCNQNRIEERSQTVKCSCLSGQVAGTTRAKPSCVDASIVLQRWWCQMEPCLPGEECKVLPDLSGWSCSSGHKVKTTKVTR

SEQ ID NO: 122 - protein, 93 aa, synthetic construct
  REGION 1..93: note = TAFA3_Rattus norvegicus
VKQGTCEVIAAHRCCNRNRIEERSQTVKCSCLSGQVAGTTRAKPSCVDASIVLQKWWCQMEPCLLGEECKVLPDLSGWSCSRGHKVKTTKVTR

SEQ ID NO: 123 - protein, 93 aa, synthetic construct
  REGION 1..93: note = TAFA3_Mus musculus_isoform1
VKQGTCEVIAAHRCCNRNRIEERSQTVKCSCLSGQVAGTTRAKPSCVDASIVLQKWWCQMEPCLLGEECKVLPDLSGWSCSSGHKVKTTKVTR

SEQ ID NO: 124 - protein, 93 aa, synthetic construct
  REGION 1..93: note = TAFA3_Gallus gallus
VEPGTCEVIAAHRCCNKNKIEERSQTVKCSCFPGQVAGTTRAAPSCVDASIVLQKWWCQMEPCLAGEECKVLPDLSGWSCSSGNKVKTTKVTR

SEQ ID NO: 125 - protein, 93 aa, synthetic construct
  REGION 1..93: note = TAFA3_Varanus komodoensis_isoform2
IEPGTCEVIAAHRCCNKNKIEERSQTVKCSCFPGQVAGTTRAAPSCVDASIVLQKWWCQMQPCLEGEECKVLPDLSGWSCSTGNKVKTTKVTR

SEQ ID NO: 126 - protein, 93 aa, synthetic construct
  REGION 1..93: note = TAFA3_Podarcis muralis
IEPGTCEVIAAHRCCNKNKIEERSQTVKCSCFPGQVAGTTHAAPSCVDASIVLQKWWCQMQPCVEGEECKVLPDLSGWSCSTGNKVKTTKVTR

SEQ ID NO: 127 - protein, 93 aa, synthetic construct; identical to SEQ ID NO: 125
  REGION 1..93: note = TAFA3_Sceloporus undulatus

SEQ ID NO: 128 - protein, 93 aa, synthetic construct
  REGION 1..93: note = TAFA3_Xenopus tropicalis_isoform2
VEPGTCEVIAAHRCCNKNKIEERSQTVKCSCFPGQVAGTTRAAPSCVDASIVIQKWWCQMEPCLEGEDCKVLPDLSGWSCSTGNKVKTTKVTR

SEQ ID NO: 129 - protein, 93 aa, synthetic construct
  REGION 1..93: note = TAFA3_Danio rerio
VKAGTCEVIAAHRCCNRNKIEERSQTVKCSCFPGQVAGTTRAAPSCVDASIVAQKWWCQMQPCVDGEECKVLPDLTGWSCSTGNKVKTTKVTR

SEQ ID NO: 130 - protein, 93 aa, synthetic construct; identical to SEQ ID NO: 87
  REGION 1..93: note = TAFA4_Macaca fascicularis_isoform2

SEQ ID NO: 131 - protein, 93 aa, synthetic construct; identical to SEQ ID NO: 87
  REGION 1..93: note = TAFA4_Sus scrofa_isoform2

SEQ ID NO: 132 - protein, 93 aa, synthetic construct
  REGION 1..93: note = TAFA4_Oryctolagus cuniculus_isoform4
IKPGTCEVVAVHRCCNKNRIEERSQTVKCSCFPGQVAGTTQAQPSCVEASIVAQKWWCHMNPCLEGEDCKVLPDYSGWSCSSGNKVKTTKVTR

SEQ ID NO: 133 - protein, 93 aa, synthetic construct
  REGION 1..93: note = TAFA4_Rattus norvegicus
IKQGTCEVVAVHRCCNKNRIEERSQTVKCSCFPGQVAGTTRAQPSCVEASIVIEKWWCHMDPCLEGEDCKVLPDSSGWSCSSGNKVKTTKVTR

SEQ ID NO: 134 - protein, 93 aa, synthetic construct
  REGION 1..93: note = TAFA4_Mus musculus
IKPGTCEVVAVHRCCNKNRIEERSQTVKCSCFPGQVAGTTRAQPSCVEAAIVIEKWWCHMNPCLEGEDCKVLPDSSGWSCSSGNKVKTTKVTR

SEQ ID NO: 135 - protein, 93 aa, synthetic construct
  REGION 1..93: note = TAFA4_Gallus gallus
VKQGTCEVVAVHRCCNKNRIEERSQTVKCSCFPGQVAGTTRAQPSCVEASIVLQKWWCHMNPCLDGEDCKVLPDYSGWSCSSGNKVKTTKVTR

SEQ ID NO: 136 - protein, 93 aa, synthetic construct
  REGION 1..93: note = TAFA4_Varanus komodoensis_isoform2
VKQGTCEVVAVHRCCNKNRIEERSQTVKCSCLPGQVAGTTRAQPSCVEAAIVVQKWWCHMNPCLEGEECKVLPDYSGWSCSSGNKVKTTKVTR

SEQ ID NO: 137 - protein, 93 aa, synthetic construct
  REGION 1..93: note = TAFA4_Podarcis muralis
VKQGTCEVVAVHRCCNKNRIEERSQTVKCSCFPGQVAGTTRAQPSCVEAAIVIQKWWCHMNPCLDGEDCKVLPDYSGWSCSSGNKVKTTKVTR

SEQ ID NO: 138 - protein, 93 aa, synthetic construct
  REGION 1..93: note = TAFA4_Sceloporus undulatus
VKQGTCEVVAVHRCCNKNRIEERSQTVKCSCFPGQVAGTTRSQPSCVEAAIVIQKWWCHMNPCLEGEECKVLPDYSGWSCSSGNKVKTTKVTR

SEQ ID NO: 139 - protein, 93 aa, synthetic construct
  REGION 1..93: note = TAFA4_Gekko japonicus
VKQGTCEVVAVHLCCNKNRIEELSQTGNCSCLPGQVAGTTRTQPSCVEAAIVIQKWWCQMSPCLEGEECKVLPDSSGWSCSSGNKVKTTKVTR

SEQ ID NO: 140 - protein, 93 aa, synthetic construct
  REGION 1..93: note = TAFA4_Xenopus tropicalis
VKQGTCEVVALHRCCNKNRIEERSQTVKCSCFPGQVAGTTRAQPSCVEASIVIQKWWCHMNPCMEGEECKVLPDLTGWSCSSGNKIKTTKVTR

SEQ ID NO: 141 - protein, 93 aa, synthetic construct
  REGION 1..93: note = TAFA4_Danio rerio
VKQGTCEVVAIHRCCNKNKIEERSQTVKCSCFPGQVAGTTRAQPSCVEASIVLQKWWCQMHPCLDGEECKALPDLTGWSCSTGNKVKTTKVTR

SEQ ID NO: 142 - protein, 8 aa, synthetic construct
  REGION 1..8: note = Formula 1
  VARIANT 1: note = Xaa is E, D, P, L or A
  VARIANT 4: note = Xaa is D or E
  VARIANT 7: note = Xaa is T, V, I or A
XGEXCKXL

SEQ ID NO: 143 - protein, 22 aa, synthetic construct
  REGION 1..22: note = Formula 2
  VARIANT 3: note = Xaa is I, E, A, L or V
  VARIANT 4: note = Xaa is Q, E or G
  VARIANT 5: note = Xaa is K or R
  VARIANT 9: note = Xaa is E, H or Q
  VARIANT 11: note = Xaa is E, Q, N, D, S or H
  VARIANT 14: note = Xaa is L, M or V
  VARIANT 15: note = Xaa is E, D, P, L or A
  VARIANT 18: note = Xaa is D or E
  VARIANT 21: note = Xaa is T, V, I or A
IVXXXWWCXMXPCXXGEXCKXL

SEQ ID NO: 144 - protein, 29 aa, synthetic construct
  REGION 1..29: note = Formula 3
  VARIANT 1: note = Xaa is E, D, P, L or A
  VARIANT 4: note = Xaa is D or E
  VARIANT 7: note = Xaa is T, V, I or A
  VARIANT 11: note = Xaa is Y, S or L
  VARIANT 12: note = Xaa is S or T
  VARIANT 18: note = Xaa is S or T
  VARIANT 22: note = Xaa is V or I
XGEXCKXLPDXXGWSCSXGNKXKTTKVTR

SEQ ID NO: 145 - protein, 17 aa, synthetic construct
  REGION 1..17: note = Formula 4
  VARIANT 2: note = Xaa is Q or K
  VARIANT 8: note = Xaa is R, H or Q
  VARIANT 9: note = Xaa is A, N, S or T
  VARIANT 10: note = Xaa is R, A, Q, K, or T
  VARIANT 15: note = Xaa is D or E
  VARIANT 16: note = Xaa is A or does not exist
  VARIANT 17: note = Xaa is S, A or does not exist
GXVAGTTXXXPSCVXXX

SEQ ID NO: 146 - protein, 32 aa, synthetic construct
  REGION 1..32: note = Formula 5
  VARIANT 1: note = Xaa is R or K
  VARIANT 5: note = Xaa is R or L
  VARIANT 9: note = Xaa is V or G
  VARIANT 10: note = Xaa is K or N
  VARIANT 14: note = Xaa is F or L
  VARIANT 15: note = Xaa is P or S
  VARIANT 17: note = Xaa is Q or K
  VARIANT 23: note = Xaa is R, H or Q
  VARIANT 24: note = Xaa is A, N, S or T
  VARIANT 25: note = Xaa is R, A, Q, K or T
  VARIANT 30: note = Xaa is D or E
  VARIANT 31: note = Xaa is A or does not exist
  VARIANT 32: note = Xaa is S, A or does not exist
XIEEXSQTXXCSCXXGXVAGTTXXXPSCVXXX

SEQ ID NO: 147 - protein, 31 aa, synthetic construct
  REGION 1..31: note = Formula 6
  VARIANT 2: note = Xaa is Q or K
  VARIANT 8: note = Xaa is R, H or Q
  VARIANT 9: note = Xaa is A, N, S or T
  VARIANT 10: note = Xaa is R, A, Q, K or T
  VARIANT 15: note = Xaa is D or E
  VARIANT 16: note = Xaa is A or does not exist
  VARIANT 17: note = Xaa is S, A or does not exist
  VARIANT 20: note = Xaa is I, A, V or L
  VARIANT 21: note = Xaa is Q or E
  VARIANT 26: note = Xaa is H or Q
  VARIANT 28: note = Xaa is N, D, S or H
  VARIANT 31: note = Xaa is L or M
GXVAGTTXXXPSCVXXXIVXXKWWCXMXPCX

SEQ ID NO: 148 - protein, 35 aa, synthetic construct
  REGION 1..35: note = Human TAFA4 fragment 1
HQIKQGTCEVVAVHRCCNKNRIEERSQTVKCSCFP

SEQ ID NO: 149 - protein, 20 aa, synthetic construct
  REGION 1..20: note = Human TAFA4 fragment 4
HQIKQGTCEVVAVHRCCNKN

SEQ ID NO: 150 - protein, 17 aa, synthetic construct
  REGION 1..17: note = Human TAFA4 fragment 6
FPGQVAGTTRAQPSCVE

SEQ ID NO: 151 - protein, 21 aa, synthetic construct
  REGION 1..21: note = Human TAFA4 fragment 8
PDYSGWSCSSGNKVKTTKVTR

SEQ ID NO: 152 - protein, 28 aa, synthetic construct
  REGION 1..28: note = Human TAFA1 fragment 3
EGEECKTLPDNSGWMCATGNKIKTTRIH

SEQ ID NO: 153 - protein, 28 aa, synthetic construct
  REGION 1..28: note = Komodo dragon TAFA1 fragment 3
EGEECKTLPDNSGWMCATGNKVKTTRIH

SEQ ID NO: 154 - protein, 28 aa, synthetic construct
  REGION 1..28: note = Frog_isoform2 TAFA1 fragment 3
EGEECKTLPDNSGWMCATGNKIKTTRFQ

SEQ ID NO: 155 - protein, 29 aa, synthetic construct
  REGION 1..29: note = Fish_isofrom1 TAFA1 fragment 3
EGEECKTLPDNSGWMCYSGNKIKTTRGNI

SEQ ID NO: 156 - protein, 29 aa, synthetic construct
  REGION 1..29: note = Fish_isofrom2 TAFA1 fragment3
EGEECKTLPDNSGWMCYSGNKIKTTRNTH

SEQ ID NO: 157 - protein, 29 aa, synthetic construct
  REGION 1..29: note = Human TAFA2 fragment 3
EGEECKVLPDRKGWSCSSGNKVKTTRVTH

SEQ ID NO: 158 - protein, 29 aa, synthetic construct
  REGION 1..29: note = Rat isoform1 TAFA2 fragment 3
EGEECKVLPDRKGWSCSSGNKVKTTRANV

SEQ ID NO: 159 - protein, 29 aa, synthetic construct
  REGION 1..29: note = Chicken isoform2 TAFA2 fragment 3
EGEECKVLPDRKGWSCSSGNKVKTTRVTR

SEQ ID NO: 160 - protein, 29 aa, synthetic construct
  REGION 1..29: note = Komodo dragon TAFA2 fragment 3
EGEECKVLPDRKGWSCSSGNKVKTTRVSK

SEQ ID NO: 161 - protein, 27 aa, synthetic construct
  REGION 1..27: note = Wall lizard TATA2 fragment 3
EGEECKVLPDRKGWSCSSGNKVKTTRM

SEQ ID NO: 162 - protein, 28 aa, synthetic construct
  REGION 1..28: note = Gecko TAFA2 fragment 3
EGEECKVLPDRKGWSCSSGNKVKTTRAN

SEQ ID NO: 163 - protein, 29 aa, synthetic construct
  REGION 1..29: note = Frog TAFA2 fragment 3
EGEECKILPDQKGWSCASGNKVKTTKVTR

SEQ ID NO: 164 - protein, 29 aa, synthetic construct
  REGION 1..29: note = Fish TAFA2 fragment 3
DGEECKVLPDLKGWSCSTGNKVKTTKVTR

SEQ ID NO: 165 - protein, 29 aa, synthetic construct
  REGION 1..29: note = Human TAFA3 fragment 3
PGEECKVLPDLSGWSCSSGHKVKTTKVTR

SEQ ID NO: 166 - protein, 29 aa, synthetic construct
  REGION 1..29: note = Rat TAFA3 fragment 3
LGEECKVLPDLSGWSCSRGHKVKTTKVTR

SEQ ID NO: 167 - protein, 29 aa, synthetic construct
  REGION 1..29: note = Mouse TAFA3 fragment 3
LGEECKVLPDLSGWSCSSGHKVKTTKVTR

SEQ ID NO: 168 - protein, 29 aa, synthetic construct
  REGION 1..29: note = Chicken TAFA3 fragment 3
AGEECKVLPDLSGWSCSSGNKVKTTKVTR

SEQ ID NO: 169 - protein, 29 aa, synthetic construct
  REGION 1..29: note = Komodo dragon TAFA3 fragment 3
EGEECKVLPDLSGWSCSTGNKVKTTKVTR

SEQ ID NO: 170 - protein, 29 aa, synthetic construct
  REGION 1..29: note = Frog TAFA3 fragment 3
EGEDCKVLPDLSGWSCSTGNKVKTTKVTR

SEQ ID NO: 171 - protein, 29 aa, synthetic construct
  REGION 1..29: note = Fish TAFA3 fragment 3
DGEECKVLPDLTGWSCSTGNKVKTTKVTR

SEQ ID NO: 172 - protein, 31 aa, synthetic construct
  REGION 1..31: note = Human TAFA1 fragment 2
GKVAGTTRNRPSCVDASIVIGKWWCEMEPCL

SEQ ID NO: 173 - protein, 31 aa, synthetic construct
  REGION 1..31: note = Fish TAFA1 fragment 2
GKVAGTTRNKPSCVDASIVIGKWWCEMEPCL

SEQ ID NO: 174 - protein, 31 aa, synthetic construct
  REGION 1..31: note = Human TAFA2 fragment 2
GQVAGTTRAAPSCVDASIVEQKWWCHMQPCL

SEQ ID NO: 175 - protein, 31 aa, synthetic construct
  REGION 1..31: note = Gecko TAFA2 fragment 2
GQVAGTTRAAPSCVDASIVEQKWWCQMQPCL

SEQ ID NO: 176 - protein, 31 aa, synthetic construct
  REGION 1..31: note = Frog TAFA2 fragment 2
GQVAGTTRATPSCVDASIVEQKWWCHMQPCL

SEQ ID NO: 177 - protein, 31 aa, synthetic construct
  REGION 1..31: note = Fish TAFA2 fragment 2
GQVAGTTRAAPSCVDASIVAQKWWCQMQPCM

SEQ ID NO: 178 - protein, 31 aa, synthetic construct
  REGION 1..31: note = Human TAFA3 fragment 2
GQVAGTTRAKPSCVDASIVLQRWWCQMEPCL

SEQ ID NO: 179 - protein, 31 aa, synthetic construct
  REGION 1..31: note = Pig TAFA3 fragment 2
GQVAGTTRAKPSCVDASIVLQKWWCQMEPCL

SEQ ID NO: 180 - protein, 31 aa, synthetic construct
  REGION 1..31: note = Chicken TAFA3 fragment 2
GQVAGTTRAAPSCVDASIVLQKWWCQMEPCL

SEQ ID NO: 181 - protein, 31 aa, synthetic construct
  REGION 1..31: note = Komodo dragon TAFA3 fragment 2
GQVAGTTRAAPSCVDASIVLQKWWCQMQPCL

SEQ ID NO: 182 - protein, 31 aa, synthetic construct
  REGION 1..31: note = Wall lizard TAFA3 fragment 2
GQVAGTTHAAPSCVDASIVLQKWWCQMQPCV

SEQ ID NO: 183 - protein, 31 aa, synthetic construct
  REGION 1..31: note = Frog TAFA3 fragment 2
GQVAGTTRAAPSCVDASIVIQKWWCQMEPCL

SEQ ID NO: 184 - protein, 31 aa, synthetic construct
  REGION 1..31: note = Fish TAFA3 fragment 2
GQVAGTTRAAPSCVDASIVAQKWWCQMQPCV